European Patent Application EP 4 628 588 A1, published October 8, 2025. Title: Novel Fumonisin degrading enzyme and use thereof. Applicant: CJ CheilJedang Corporation. Application KR. The sequence listing filed with the application follows.

SEQUENCE LISTING (12 sequences)

SEQ ID NO: 1 - protein, 488 aa, synthetic construct
  source 1..488: note = EFB1-9
MEPVIVQTSTGALAGSGGDIRVFKGVPFGAPPIGALRWRPPEPPTPWQGVRDATQFGADCMQKRLPDTRAPGVSEDCLTLNIWAPAQNSGGALPVMVWVYGGGFVDGSASLPIYDGEALARKGVVVVTVNYRTGVFGFLAHPALAAESPHHSAGNYGILDVIAALRWLKSNVAAFGGDPNRVTVFGESAGASLLDMVLVSPLSEGLVHGAILESPGAMRPLSSLTDASEIGKIVGPDIAAMREMSAEQVLAMTDRIVPAVRRLTTPRALGPILDGWVVPRTDTAAFATGEIHRVPLIVGGNSDEGRLFVRNWPIHTVDEARAYADTNFGASAGELMALYKFDKDAAVPSALSYAFGDTQFNYGVRGLARGMSKVQPKTFRYLFTRSPGGVPPAPTHSEEIDYALANLGAHRFIPRGAFDATDRTLSAAMADAWVRFASTGDPNGGMLPHWPAYDGESDPYLEFGDSIRVGQGYRTTYLDFVESFLTKP

SEQ ID NO: 2 - DNA, 1464 bp, synthetic construct
  source 1..1464: mol_type = other DNA; note = EFB1-9
atggagcccgtcatcgttcaaacttcaactggagctcttgcgggcagcggcggggatataagagtattcaaaggggtgccattcggtgcgcctccgattggagcattaagatggagaccacctgaaccccccacgccttggcagggtgtacgtgacgctacgcagttcggggctgactgtatgcagaaaagactgccagacacgcgcgcaccgggcgtatcagaggactgcttgacattaaatatctgggcaccagcccagaatagtggcggcgcactgcccgttatggtctgggtctatgggggcggatttgtcgacggttcagcatctcttcccatctacgacggggaggcattagctcgcaaaggcgttgtcgttgttacggttaactatagaacaggtgtgttcgggtttttagctcatcccgccttagcggcggagagtccgcatcatagtgcggggaactacggtatcttagacgtgattgccgcgctgagatggttaaaatcgaacgtggcggccttcggaggggaccctaatcgggtcacggtatttggagaaagtgcaggagcttcattgttggatatggtgttggtttcgccgctgagtgaaggcttggtacatggcgccatactggaatctccgggggcaatgcgtccactttcgtcattaaccgacgcgtccgaaatcggtaaaatagtggggccagatatagcggccatgcgtgaaatgtcggcggaacaagtacttgctatgactgatcgtattgtcccggctgtccgccgtctgacgacaccccgtgcgttaggcccaatcttggacggttgggtagtaccacggacagacacggcggcgtttgcgactggcgagatacacagagtaccgcttattgttggcggaaattcagatgaagggcggctgttcgttcggaattggccaatccatactgttgatgaagcacgcgcgtatgcggacacgaatttcggagcgagtgcgggagagctgatggccttatacaaattcgacaaagacgccgcagtgccatccgcgttaagttacgcattcggggacacgcaatttaattatggtgtccgtgggctggcacgcggcatgtccaaggtgcagccaaaaacgtttcgctatttgtttacccgttcgccaggcggggttcccccagcgcccacgcactccgaggaaatcgactatgccttagccaacctgggcgctcatcggtttatccctcggggcgccttcgatgcaaccgaccgcaccttaagtgcagcgatggcggacgcgtgggtccggtttgcctccactggagaccctaatgggggcatgttgcctcattggcctgcgtatgatggcgaatcggatccctaccttgagttcggcgattctataagagtaggccaaggctatagaacaacgtacttagacttcgtcgagagtttcttaaccaaaccg

SEQ ID NO: 3 - protein, 494 aa, synthetic construct
  source 1..494: note = CB1
MEPVIVQTSTGALAGSGGDIRVFKGVPFGAPPIGALRWRPPEPPTPWQGVRDATQFAPDCIGNERLREGSRAAGTSEDCLYLNIWAPAQNSGGALPVMVWVYGGGFSGGSGAVPYYDGEALARKGVVVVTFNYRAGILGFLAHPALAAESPHHSAGNYGILDVIAALRWLKSNVAAFGGDPNRVTVFGESAGASLLDMVLVSPLSEGLVHGAILQSPGAMRPLATLSESEANGLELGADISALRRADAGELTKIAQSRIPMSRQFTKPRPMGPILDGWVVPRTDTAAFATGEIHRVPLIVGGNADEGRAFTDRLPVKTVLEYRAYLTEQFGDEADAWERCYPANSDADVPAAVARLFGDSQFNYGVRGLARGMSKVQPKTFRYLFTGIPGAGRRPATHGDEIPYVFANLGPSSVSMFGSLEGGAGASDIKLATEMSAAWVRFASTGDPNGGMLPHWPAYDGESDPYLEFGSSIRVGQGYRTTYLDFVESFLTKP

SEQ ID NO: 4 - DNA, 1482 bp, synthetic construct
  source 1..1482: mol_type = other DNA; note = CB1
atggaacctgtgatcgtccaaaccagtacgggagcattggcagggtccggcggcgacatacgcgtcttcaagggggtaccgttcggggcacctcccataggggcattaagatggcggccaccggagccacctacgccgtggcagggcgtcagagatgccacacagttcgcccccgactgcatcggtaatgaacggcttcgcgaagggtcaagagctgctggcacgtcggaagattgcctttatttgaatatttgggcaccagcccaaaattcgggtggggctctgccggttatggtatgggtatatggcggggggttttctggtggaagcggagcagttccctactacgacggtgaagccctggctcgcaagggagtagttgttgttacgttcaattaccgcgctgggatcttaggttttttggcccacccagcgttggctgctgaatctcctcaccactcagcagggaattacggtattttggatgtaatagccgcgttaagatggttgaaatctaacgtagcggcttttggaggggaccccaatagagtaactgtatttggtgaaagcgctggagccagcctgcttgatatggtgctggtgtcgccattatcggaagggttggtacatggggccatattacagagtcctggggcaatgcggcctcttgcaacgttgtcggagtccgaggccaacggcttggaactgggagccgatatctccgcactgcgtcgtgccgacgctggggagttaacaaagatagcccagtcacggatccccatgagccgtcaattcacgaaaccccgtccgatggggcccatccttgatggttgggtagtcccgcgtacggatactgctgcttttgccaccggagagattcatcgcgtccccctgattgtgggcgggaacgctgacgagggacgcgcatttaccgatagattgcccgtaaaaacggtgttggagtaccgcgcatacctgactgagcagtttggcgacgaagccgatgcatgggaacggtgctatccagccaatagcgacgcagatgtgccagccgcagtagcccgcttgttcggagatagtcaattcaattatggagttagaggcttggctcgtggtatgtcaaaggtgcagcccaagaccttccggtatttattcacaggtatccccggcgcgggtcggcgtccggcgacacatggagacgagatcccttacgtgtttgctaatttgggtccttccagtgtgagtatgtttggaagtttagaaggcggcgcgggtgcaagtgatatcaagctggcaaccgaaatgtcagccgcttgggtgcggttcgcgtcgacgggggatcctaacgggggtatgcttcctcactggccggcttatgatggagagtcggacccgtatttagagttcggttcgtcaatccgcgtcggccaaggataccgcacgacctatcttgactttgtcgagtcatttctgactaagcct

SEQ ID NO: 5 - protein, 492 aa, synthetic construct
  source 1..492: note = CB4
MEPVIVQTSTGALAGSGGDIRVFKGVPFGAPPIGALRWRPPEPPTPWQGVRDATQFGADCMQKRLPDTRAPGVSEDCLTLNIWAPAQNSGGALPVMVWVFGGGFVDGSASLPYYDGEALARKGVVVVTVNYRTGVFGFLAHPALAAESPHHSAGNYGILDVIAALRWLKSNVAAFGGDPNRVTVFGESAGASLLDMVLVSPLSEGLVHGAILQSPGAMRPLSSLTDASEIGKIVGPDIAAMREMSAEQVLAMTDRIVPAVRRLTTPRALGPILDGWVVPRTDTAAFATGEIHRVPLIVGGNADEGRLFVRNWPIHTVDEARAYADTNFGASAGELMALYKFDKDAAVPSALSYAFGDTQFNYGVRGLARGMSKVQPKTFRYLFTGIPGAGRRPATHGDEIPYVFANLGPSSVSMFGSLEGGAGASDIKLATEMSAAWVRFASTGDPNGGMLPHWPAYDGESDPYLEFGSSIRVGQGYRTTYLDFVESFLTKP

SEQ ID NO: 6 - DNA, 1476 bp, synthetic construct
  source 1..1476: mol_type = other DNA; note = CB4
atggaaccggtcatcgttcagacttcaacaggcgcactcgcgggaagcggcggtgacatccgggttttcaagggtgtgccttttggggcaccacctattggcgcacttcgttggcggccaccagaaccgcctacgccctggcaaggagtgcgggacgcaacacaatttggcgccgactgtatgcagaaacgcctgcccgataccagagcacccggggtcagcgaggactgcctgaccttgaatatttgggctccagctcaaaattcaggtggggcattgcccgtaatggtgtgggtatttggtggcggcttcgtggatggctcggctagccttccctactacgatggtgaggcgctggcccgaaagggtgttgtagtagtgacggtaaactaccgcactggagtgtttgggttccttgcccaccccgcccttgcagctgagagtcctcaccactcagccgggaattacggaatcttagacgttatcgcagcccttcgttggcttaagtcaaatgttgcagcattcggtggtgacccaaaccgcgtcacagttttcggagagagcgctggcgcgtctctgttggatatggttctggtgagcccgttatccgagggattagttcacggcgcgattttacaatccccaggcgcgatgcgccccctttcgtcgctgacagatgcgagcgagattggcaagatcgtaggacctgacatagccgcgatgcgtgagatgtcagctgagcaagtacttgccatgaccgacagaatagtaccagctgtacgccgtctgactaccccacgtgctttaggtccaatcctggatgggtgggtggttccgcgtacggatactgctgcttttgctacgggtgagattcatcgtgttccgttaatagtcggtgggaatgccgacgaaggtcgtctgtttgtccggaactggccaatacatacagtagacgaggcacgggcctatgccgacactaactttggggctagtgccggtgaacttatggccctgtataagttcgacaaggatgcggcagtgccatccgctttgagttacgcgtttggtgatacgcaatttaactacggtgttcgtgggcttgcccgaggcatgagcaaagtgcaaccgaagactttccgttatctgttcaccgggatccctggtgccggtcgacgtccggctactcatggcgacgaaataccgtatgtgttcgcgaacttaggccccagcagtgttagtatgttcggatcattggagggaggagcgggcgctagtgatattaagctggcgacagaaatgagtgcagcttgggtccgtttcgcttcaactggggacccaaacggtgggatgttaccgcactggccagcgtacgacggtgagagcgatccatatttggagttcggcagttctatccgggtcggccaagggtaccgcactacttacttggattttgtggagtcgttccttacgaagccg

SEQ ID NO: 7 - DNA, 36 bp, synthetic construct
  source 1..36: mol_type = other DNA
cggcagccatatggagcccgtcatcgttcaaacttc

SEQ ID NO: 8 - DNA, 39 bp, synthetic construct
  source 1..39: mol_type = other DNA
tcgagtgcggccgctcacggtttggttaagaaactctcg

SEQ ID NO: 9 - DNA, 36 bp, synthetic construct
  source 1..36: mol_type = other DNA
ggcagccatatgatggaacctgtgatcgtccaaacc

SEQ ID NO: 10 - DNA, 44 bp, synthetic construct
  source 1..44: mol_type = other DNA
tcgagtgcggccgctcaaggcttagtcagaaatgactcgacaaa

SEQ ID NO: 11 - DNA, 35 bp, synthetic construct
  source 1..35: mol_type = other DNA
ggcagccatatgatggaaccggtcatcgttcagac

SEQ ID NO: 12 - DNA, 38 bp, synthetic construct
  source 1..38: mol_type = other DNA
tcgagtgcggccgctcacggcttcgtaaggaacgactc